European Patent Application EP 4 756 015 A1, published June 10, 2026. Title: BIOENZYME FOR CATALYZING HYDROXYLATION OF C9 POSITION IN TAXANE COMPOUND, AND NUCLEIC ACID MOLECULE, BIOLOGICAL MATERIAL AND USE THEREOF. Applicant: AGRICULTURAL GENOMICS INSTITUTE AT SHENZHEN, CHINESE ACADEMY OF AGRICULTURAL SCIENCES (SHENZHEN BRANCH, GUANGDONG LABORATORY FOR LINGNAN MODERN AGRICULTURE). The sequence listing filed with the application follows.

SEQUENCE LISTING (35 sequences)

SEQ ID NO: 1 - protein, 501 aa, unidentified
  source 1..501: note = T9H1 protein sequence
MDSLSFLKSMEAKFGQVIHRDQSSSTALLSLAFTAALAIFLVLLFRFKSRPSTNFPPGNFGFPFIGETIQFLRALRSESPHMFFDERLKKFGRVFKTSLTGHPTAVFCGPAGNRFIYSNEHKLVQSSGPNSFVKLVGQQSIVTKTGEEHRIFRGVLNEFLGPHALQSYTPKMSSKIQENINKHWKGKDEVNMLPSIRQLVFSISSSLFFDINDEDQQEQLKTLLETILVGTLSVPLDIPGSNFRKALRARSKLDEILSRLIESRRKDMRSGIASTSKNLLSVLLAFKDERGNPLTDTEILDNFSFMLHASYDTTVSPTVCIFKLLSANPECYEKVVQEQLGILGNKKDGEEICWNDLKAMKYTWQAAQETMRLFPPAFGSFRKVIADIHHDGYIIPKGWKAMVTNYSTSRKEEYFDEPDKFKPSRFGDGKYVAPYTFLPFGAGIRICPGWEFAKLEMLLFIHHFVKNFSGYLPLDTKEKISGDPFPPLPKNGFPIKLFPRT

SEQ ID NO: 2 - protein, 489 aa, unidentified
  source 1..489: note = T9H2 protein sequence
MDCFNFLTSMESSTALRLSLAFTAAVGIFLLLLFHYKRRPSINLPPGNFGFPFIGETIQFLRGLRSESPHVFFDERLKKFGSVFKTSLTGHPTAVFCGPAGNRLIFSNEDKLVQSSGPNSFVKLFGQQSIVSKTGEEHRIFRGALAQFLGPHALQSYTPKINSKIQENIDKKWKGKDEVKMLPLIRGLIFSIASSLFFDINDEDQQEQLHTLLETILLGTLSIPLDFPGSNFRKALKARSKLDEILSCLIKSRRKDMRSGIASTNQNLLSVLLTFKDERGNPLTDMEILDNFSVMLHASYDTTVSPTILLFKLLSANPECYEKVVQEQLGILGDKDGEEIVWNDLKCMKYTWQVVQETMRIFPPTFGSFRKVIADIHHDGYTIPKGWRVLVTNHSTSGKEEYFDEPDKFKPSRFEDGKYVAPYTFLPFGAGIRICPGWEFAKLEMLLFIHHFVKHFSGYIPIDTKEKVSGDPFPPLPNNGFPIKLLPRT

SEQ ID NO: 3 - protein, 499 aa, unidentified
  source 1..499: note = T9H3 protein sequence
MDRFNLLRGIVSNLGEVIQLDSSPAIISLTLAAILGIIVLFIFRYNHRSSVKLPPGNLGFPFIGETVPFLRALRSETPQTFFDGRMKKFGPVFLTSLIGHPTVVFCGPAGNRLLLSNEDKLVNMTSPKSSRKVFGQNSIVTKRGEEHRIFRAALIRFLRPQAIQSYIGRMNSKVERHINEKWKGKDEVKALPLIRDLIFSIASSLFFDINDEHQQKRLHHLLETVLMGSMSVPLDFPGTPFRKAVQARSKLDEVLSCLIKSRRNDLRSGIASEDQDLLSVLLTFKDERGNPLADNEILDNFSVILHASYDTTVSPTVLLFKFLFSNPECYEKVVQEQLGIHGNKKEGEEINWNDLKAMKYTWQVVQETMRIFPPAFGAFRQAITDIHYDGYTVPKGYNILWTPYATHVKEEYFNEADKFMPSRFEEGKYVTPYTYLPFGAGLRVCPGWEFAKAEMLLIVHHFVRNFSSFFPVDPNEKISGDPFPPLPTNGFSMKLFPRS

SEQ ID NO: 4 - protein, 501 aa, unidentified
  source 1..501: note = T9H4 protein sequence
MDSLSFLKSMEAKFGQVIHRDQSSSTALLSLAFTAALAIFLVLLFRFKSRPSTNFPPGNFGFPFIGETIQFLRALRSESPHMFFDERLKKFGRVFKTSLTGHPTAVFCGPAGNRFIYSNEHKLVQSSGPNSFVKLVGQQSIVTKTGEEHRIFRGVLNEFLGPHALQSYTPKMSSKIQENINKHWKGKDEVNMLPSIRQLVFSISSSLFFDINDEDQQEQLKTLLETILVGTLSVPLDIPGSNFRKALRARSKLDEILSRLIESRRKDMRSGIASTSKNLLSVLLAFKDERGNPLTDTEILDNFSFMLHASYDTTVSPTVCIFKLLSANPECYEKVVQEQLGILGNKKDGEEICWNDLKAMKYTWQAAQETMRLFPPAFGSFRKVIADILHDGYIIPKGWKAMVTNYSTSRKEEYFDEPDKFKPSRFGEGKYVAPYTFLPFGAGIRICPGWEFAKLEMLLFIHHFVKNFSGYLPLDTKEKISGDPFPPLPKNGFPIKLFPRT

SEQ ID NO: 5 - protein, 499 aa, unidentified
  source 1..499: note = T9H5 protein sequence
MDRFNLLRGIVSNLGEVIQLDSSPAFISLTLAAILGIIVLFIFRYNHRSSVKLPPGNLGFPFIGETIPFLRALRSETPQTFFDGRMKKFGPVFLTSLIGHPTVVFCGPAGNRLLLSNEDKLVNMTSPKSSRKVFGQNSIVTKRGEEHRIFRAALTRFLRPQAIQSYIGRMNSKVERHINEKWKGKDEVKALPLIRDLIFSIASSLFFDINDEHQQKRLHHLLETVLMGSMSVPLDFPGTPFRKAVQARSKLDEILSCLIKSRRNDLRSGIASEDQDLLSVLLTFKDERGNPLADNEILDNFSVILHASYDTTVSPTVLLFKFLFSNSECYEKVVQEQLGIHGNKKEGEEINWNDLKAMKYTWQVVQETMRIFPPAFGAFRQAITDIHYDGYTVPKGYNILWTPYATHVKEEYFNEADKFMPSRFEEGKYVTPYTYLPFGAGLRVCPGWEFAKAEMLLIVHHFVRNFSSFFPVDPNEKISGDPFPPLPTNGFSMKLFPRS

SEQ ID NO: 6 - protein, 501 aa, unidentified
  source 1..501: note = T9H6 protein sequence
MDSFSFLKSMEAKFGQVIHRDQSSSTALLSLAFTAAVAIFLVLLFRFKSRPSTNFPPGNFGFPFIGETIQFLRALRSESPHMFFDERLKKFGRVFKTSLTGHPTAVFCGPAGNRFIYSNEHKLVQSSGPNSFVKLVGQQSIVTKTGEEHRIFRGVLNEFLGPHALQSYTPKMSSKIQENINKHWKGKDEVNMLPSIRQLVFSISSSLFFDINDEDQQEQLKTLLETILVGTLSVPLDIPGSNFRKALRARSKLDEILSRLIESRRKDMRSGIASTSKNLLSVLLAFKDERGNPLTDTEILDNFSFMLHASYDTTVSPTVCIFKLLSANPECYEKVVQEQLGILGNKKDGEEICWNDLKAMKYTWQAAQETMRLFPPAFGSFRKVIADIHHDGYIIPKGWKAMVTNYSTSRKEEYFDEPDKFKPSRFGDGKYVAPYTFLPFGAGIRICPGWEFAKLEMLLFIHHFVKNFSGYLPLDTKEKISGDPFPPLPKNGFPIKLFPRT

SEQ ID NO: 7 - protein, 499 aa, unidentified
  source 1..499: note = T9H7 protein sequence
MDRFNFVRDIVANLGEVIQLESSPAIISLTLAAILGIILLFIFRYNNRSSVKLPPGNLGFPFIGETIPFLRALRSETPQTFFDGRMKKFGPVFLTSLIGHPTVVFCGPAGNRLLLSNEDKLVNMTSPKSSRKVFGQNSIVTKRGEEHRIFRAALARFLRPQAIQSYIGRMNSKVERHINEKWKGKDEVKALPLIRYLIFSIASSLFFDINDEHQQKRLHHLLETVLMGSMSVPLDFPGTPFRKAVQARSKLDEILSCLIKSRRNDLRSGIASEDQDLLSVLLTFKDERGNPLADNEILDNFSVILHASYDTTVSPSVLLFKFLFSNPECYEKVVQEQLGIHGNKKEGEEINWNDLKAMKYTWQVVQETMRIFPPAFGAFRQAITDVHYDGYTVPKGYNILWTPYATHVKEEYFNEADKFMPSRFEEGKYVAPYTYLPFGAGLRVCPGWEFAKAEMLLIVHHFVRNFSSFFPVDPNEKISGDPFPPLPTNGFSMKLFPRS

SEQ ID NO: 8 - protein, 501 aa, unidentified
  source 1..501: note = T9H8 protein sequence
MDSFSFLKSMEAKFGQVIHRDQSSSTVLLSLAFTAAVAIFLVLLFRFKSRPSTNFPPGNFGFPFIGETIQFLRALRSESPHRFFDERLKKFGNVFKTSLTGHPTAVFCGPAGNRFIYSNEHKLVQSSGPNSFVKLVGQQSIVTKTGEEHRIFRGVLNEFLGPHALQSYTPKMSSKIQENINKHWKGKDEVNMLPSIRQLVFSISSSLFFDINDEDQQEQLKTLLETILVGTLSVPLDIPGSNFRKALRARSKLDEILSRLIESRRKDMRSGIASTSKNLLSVLLAFKDERGNPLTDTEILDNFSFMLHASYDTTVSPTVCIFKLLSANPECYEKVVQEQLGILGNKKDGEEICWNDLKAMKYTWQAAQETMRLFPPAFGSFRKVIADIHHDGYIIPKGWKAMVTNYSTSRKEEYFDEPDKFKPSRFGDGKYVAPYTFLPFGAGIRICPGWEFAKLEMLLFIHHFVKNFSGYLPLDTKEKISGDPFPPLPKNGFPIKLFPRT

SEQ ID NO: 9 - protein, 499 aa, unidentified
  source 1..499: note = T9H9 protein sequence
MDRFNLLRGIVSNLGEVIQLDSSPAIISLTLAAILGIIVLFIFRYNHRSSVKLPPGNLGFPFIGETIPFLQALRSETPQTFFDGRMKKFGPVFLTSLIGHPTVVFCGPAGNRLLLSNEDKLVNMTSPKSSRKVFGQNSIVTKRGEEHRIFRAALTRFLRPQAIQSYIGRMNSKVERHINEKWKGKDEVKALPLIRDLIFSIASSLFFDINDEHQQKRLHHLLETVLMGSMSVPLDFPGTPFRKAVQARSKLDEVLSCLIKSRRNDLRSGIASEDQDLLSVLLTFKDERGNPLADNEILDNFSVILHASYDTTVSPTVLLFKFLFSNPECYEKVVQEQLGIHGNKKEGEEINWNDLKAMKYTWQVVQETMRIFPPAFGAFRQAITDIHYDGYTVPKGYNILWTPYATHVKEEYFNEADKFMPSRFEEGKYVTPYTYLPFGAGLRVCPGWEFAKAEMLLIVHHFVRNFSSFFPVDPTEKISGDPFPPLPTNGFSMKLFPRS

SEQ ID NO: 10 - protein, 492 aa, unidentified
  source 1..492: note = T9H10 protein sequence
MDSFNFPRGGVIQLGYSPAILSLTLAPILAILLLFFFRYTHRSSDKLPPGNLGFPFIGETIQLMRALRTETPQTFFDERVKKFGHVFKTSLIGYPTVVLSGPAGNRLLLSNEEKLVHSSSPKSTLKLFGQDSVLTKRGEEHRIFRAALARFLRPQALQGYVAKMNSEIQHHMNQKWKGKHQVKVLPLVRALIFNIASSFFFGITDEHLQERLHNLLEAILLGSMSVPLDFPGTRFRKALEARSKLDEILSSLIKKRRSDLLRSTSDNQDLLSVLLTFKDERGNPLTDKEILDNFSVMLHGSYETSVSPTVLVFKLLFSNPDCYEKVVQEQLGILCNKKEGEEISWNDLKTMKYTWQVVQETMRMFPPVFGSYRKAITDIHYDGYTIPKGWKIFWSPYTTHGKEEYFNEADKFMPSRFEEGKYVAPYTFLPFGAGVRVCPGWEFAKTEILLFVHHFVRTFSSYIPIDPKEKISGDPFPPLPTNGFSMKLFSRS

SEQ ID NO: 11 - protein, 492 aa, unidentified
  source 1..492: note = T9H11 protein sequence
MDSFNFPRGGVIQLGYSPAILSLTLAPILAILLLFFFRYTHRSSDKLPPGNLGFPFIGETIQLMRALRTETPQTFFDERVKKFGHVFKTSLIGYPTVVLSGPAGNRLLLSNEEKLVHSSSPKSTLKLFGQDSVLTKRGEEHRIFRAALARFLRPQALQGYVAKMNSEIQHHMNQKWKGKHQVKVLPLVRALIFNIASSFFFGITDEHLQERLHNLLEAILLGSMSVPLDFPGTRFRKALEARSKLDEILSSLIKKRRSDLLRSTSDNQDLLSVLLTFKDERGNPLTDKEILDNFSVMLHGSYETSVSPTVLVFKLLFSNPDCYEKVVQEQLGILCNKKEGEEISWNDLKTMKYTWQVVQETMRMFPPVFGSYRKAITDIHYDGYTIPKGWNIFWSPYTTHGKEEYFNEADKFMPSRFEEGKYVAPYTFLPFGAGLRVCPGWEFAKTEILLFVHHFVTTFSSYIPIDPIEKISGDPFPPLPTDGFSMKLFTRS

SEQ ID NO: 12 - protein, 501 aa, unidentified
  source 1..501: note = T9H12 protein sequence
MDSFSFLKSMEAKFGQVIHRDQSSSTALLSLAFTAAVAIFLVLLFRFKSRPSTNFPPGNFGFPFIGETIQFLRALRSESPHMFFDERLKKFGRVFKTSLTGHPTAVFCGPAGNRFIYSNEHKLVQSSGPNSFVKLVGQQSIVTKTGEEHRIFRGVLNEFLGPHALQSYTPKMSSKIQENINKHWKGKDEVNMLPSIRQLVFSISSSLFFDINDEDQQEQLKTLLETILVGTLSVPLDIPGSNFRKALRARSKLDEILSRLIESRRKDMRSGIASTSKNLLSVLLAFKDERGNPLTDTEILDNFSFMLHASYDTTVSPTVCIFKLLSANPECYEKVVQEQLGIHGNKKEGEEINWNDLKAMKYTWQAAQETMRLFPPAFGSFRKVIADIHHDGYIIPKGWKAMVTNYSTSRKEEYFDEPDKFKPSRFGDGKYVAPYTFLPFGAGIRICPGWEFAKLEMLLFIHHFVKNFSGYLPLDTKEKISGDPFPPLPKNGFPIKLFPRT

SEQ ID NO: 13 - protein, 491 aa, unidentified
  source 1..491: note = T9H13 protein sequence
MNTFSFLPPNFLGFIQLQSILFLTLLALLLLCLFRYKTPSSAVKLPPGNLGFPFIGETIPFLRALHSETPQTFFDERMKRFGNVFVTSLIGQPIVVLCGPAGNRLLLSNEDKLVEMSPPKFSLKLIGQDSLLSKREDEHRTLRAALARFLRPQALQSYMGIMSSEIEQHINEKWKVKDEVKMLPLIRGLIFSIATTLFFDINDEHLKDRLHHLLETILVGTVSLPLDFPGTSFRKAVEARSKLDEILSSLIKSRRSDLHSGIVSDGQDLLTVLLTFKDERGNSLADNEILDNFSLMLHASYETSVSPTVLMFKLLSSNPECYDKLVQEQLGILANKKEGEDISWKDVKAMKYTWQVVQETMRIFPPAFGAFRQAITDIHYDGYTVPKGYNILWTPYATHVKEEYFNEADKFMPSRFEEGKYVAPYTYLPFGAGLRVCPGWEFAKAEMLLIVHHFVRNFSSFFPVDPNEKISGDPFPPLPTNGFSMKLFPRS

SEQ ID NO: 14 - protein, 491 aa, unidentified
  source 1..491: note = T9H14 protein sequence
MNTFSFLPPNFLGFIQLQSILFLTLLALLLLCLFRYKTPSSAVKLPPGNLGFPFIGETIPFLRALHSETPQTFFDERMKRFGNVFVTSLIGQPIVVLCGPAGNRLLLSNEDKLVEMSPPKFSLKLIGQDSLLSKREDEHRTLRAALARFLRPQALQSYMGIMSSEIEQHINEKWKVKDEVKMLPLIRGLIFSIATTLFFDINDEHLKDRLHHLLETILVGTVSLPLDFPGTSFRKAVEARSKLDEILSSLIKSRRSDLHSGIVSDGQDLLTVLLTFKDERGNSLADNEILDNFSLMLHASYETSVSPTVLMFKLLSSNPECYDKLVQEQLGILANKKEGEDISWKDVKAMKYTWQVVQETMRIFPPGFGSYRKAITDIDYDGYTIPKGWTTLWTPYTTHGKEQYFHDPEQFRPSRFEEGERVAPYTFLPFGAGARICPGWEFAKTEILLFVHHFVKNFSSYHLVDPKEKVSGNPFPPLPNNGFSLKVFPRS

SEQ ID NO: 15 - DNA, 1506 bp, unidentified
  source 1..1506: mol_type = other DNA; note = T9H1 reading frame nucleotide sequence
atggattccttaagttttctaaaaagcatggaagcgaaattcggccaagtcatacaccgggatcagtcttccagtactgctcttctgtccctcgcattcacagctgctcttgccatttttcttgtgttgctctttcgatttaaaagccggccctctactaatttccctccaggaaattttggcttccctttcattggagagacgatacagttcttgcgggcacttcgatcagaatcgcctcatatgttttttgatgagagattgaagaaatttgggcgtgtattcaagacgtcattaactgggcatcccacagctgtgttctgcgggcctgcgggaaaccggtttatttactcgaatgagcacaagctggtgcagtcgtctgggcccaactccttcgtcaaactggttgggcagcaatccatcgtgaccaaaacaggagaggagcaccgcatctttcgtggtgtcctgaacgagtttctggggcctcatgccttacagagttatacgcctaaaatgagttccaaaatccaggagaatatcaataagcattggaagggtaaagatgaagtgaacatgcttccttcgataagacagctcgtcttctccatttcaagcagcttgttttttgatattaatgatgaggatcaacaggaacaacttaaaactcttttagaaactattcttgttggaactttgtcggttcccctcgacattccaggatctaattttcgtaaagctcttcgggcgcgttccaagctggatgaaattctgtctcgtttaatcgaaagcagaagaaaagatatgcgttctgggatagcttctaccagtaaaaatctactgtcggtgctgctcgccttcaaagatgaaagagggaatccattgacggacacggagatcctcgacaacttttcttttatgcttcacgcctcatacgacaccaccgtttcgcccacggtttgtatatttaagctgctctccgccaatccagaatgctatgaaaaagtagttcaagaacaattgggaatacttggcaataaaaaggacggtgaagaaatctgttggaacgatctgaaagctatgaaatatacatggcaagcagctcaagaaacaatgaggcttttccctccagcgtttggatcatttcgcaaggtcatcgccgatattcatcatgatggctatataattcccaaaggatggaaagctatggtgacaaattacagtacaagtaggaaagaagagtacttcgatgaaccagacaaattcaagccttcaagatttggggatggaaagtatgtggctccgtacacgttcttacctttcggggcaggaatacgcatatgcccaggatgggagttcgctaagttggagatgttactgttcatccatcattttgtcaaaaatttcagcggatacctcccacttgacaccaaggaaaagatttccggagatccattccctcctctccccaaaaatggatttcccattaaactatttcccagaacctaa

SEQ ID NO: 16 - DNA, 1470 bp, unidentified
  source 1..1470: mol_type = other DNA; note = T9H2 reading frame nucleotide sequence
atggattgcttcaattttctaacaagcatggagtcttccactgctcttcgactatccctcgccttcacagctgctgttggcattttccttctgttgctcttccattataaacgcaggccctctattaatcttcccccaggaaattttggcttccctttcattggagaaacgatacaattcttgcggggacttcgatcagaatcgcctcatgtgttttttgatgagagattgaagaaattcgggagtgtattcaagacgtcattaactggacatcccacagctgtgttctgcggtcctgcgggaaaccgcttaattttctcgaatgaggacaagctggtgcagtcgtcggggcccaactctttcgtcaaactgtttgggcagcaatccatcgtttccaaaacaggagaggagcatcgcatctttcgtggtgccctcgcccagtttctgggtcctcatgctttacagagttacacgcctaaaataaactccaaaatccaggagaatatcgataaaaaatggaagggcaaagatgaagtgaagatgcttcctttgataagagggctcatcttctccatcgcaagcagcttgtttttcgatattaatgatgaggatcaacaggaacaacttcatactcttttagaaactattcttctgggaacattgtcgattcctctcgactttccaggatctaattttcgtaaagctcttaaggcgcgttccaagctggatgaaattctttcttgtttgataaaaagcagaagaaaagatatgcgttctgggatagcttctaccaatcaaaatctgctgtcggtgctgctcaccttcaaagatgaaagagggaatccactgacggacatggagatcctcgacaacttttctgttatgcttcacgcctcatacgacaccactgtttcaccaacgatcttgttatttaagcttctctccgccaatccagaatgctatgaaaaagtagtccaagaacaactgggaatacttggcgataaggacggtgaagaaatcgtttggaacgatctgaaatgtatgaaatatacatggcaagtagttcaagaaacaatgaggatcttccctccaacgtttggatcatttcgcaaggttatcgccgatattcatcatgatggctacacaattccgaaaggatggagagttctggtgacaaatcacagtacaagtgggaaagaagagtacttcgatgaaccggacaaattcaagccttcaagatttgaggatggaaagtacgtagctccgtatacgttcttacctttcggggcaggcatacgcatatgcccaggatgggaattcgcaaagctggagatgttactgttcatccatcattttgttaaacatttcagtgggtacatcccaattgacaccaaggaaaaggtttccggagatccattccctcctctcccgaacaatggatttcccataaaactccttcccagaacctaa

SEQ ID NO: 17 - DNA, 1500 bp, unidentified
  source 1..1500: mol_type = other DNA; note = T9H3 reading frame nucleotide sequence
atggatcgcttcaatttgctgagaggcatagtttcaaatttaggggaagtcattcaactggactcttcccctgctattatttcccttaccctcgcagctatccttggcattattgtcctctttatcttccgttataatcaccgatcttctgttaaacttccccctggaaatttaggcttccccttcattggggagaccgtaccattcttgcgggcgcttcgatcagaaacccctcaaacattttttgatgggagaatgaagaaattcggtcctgttttcctgacatcgctaattgggcatcccacagttgtattctgcgggcctgcgggaaatcgccttcttctctccaacgaggacaaactggtaaacatgacatcgcccaagtcttccagaaaagtgtttgggcagaattccattgtgaccaaaagaggcgaggagcatcgcatcttccgtgctgcacttatccgttttttgcgtccccaagccatacagagttatattggtagaatgaattccaaagtcgaacgtcatatcaacgaaaaatggaagggaaaagacgaagtgaaggcgcttcctttgataagagacctcatcttttccattgcaagcagtctgtttttcgatataaatgatgagcaccaacagaagcgacttcatcatctgttggaaaccgttcttatgggaagtatgtctgtcccgctcgactttccaggaactccttttcgtaaagctgttcaggcgcgatcaaagctggatgaagttctttcttgtttgataaaaagcagaagaaacgatctccgttcgggcatagcttctgaagatcaagatcttctctctgtgttgctcaccttcaaagatgaaagaggaaatccactcgccgacaacgagatcctggacaacttttctgttatacttcatgcctcgtatgacaccactgtttcacccactgttttgttatttaaattcctcttctccaatcctgaatgctatgaaaaagttgttcaagagcaattgggaatccatggcaataaaaaggagggggaagaaatcaattggaacgatctgaaagctatgaaatatacatggcaagtagttcaggaaacaatgaggattttccctccagcttttggagcttttcgccaagctatcaccgatattcactacgatggctatacagttccaaagggatacaatatattatggacaccttatgctacacatgtgaaagaagagtacttcaatgaagcggacaagttcatgccttcaagattcgaggaaggcaaatatgttaccccttacacatacttgccattcggagcaggcttgcgcgtatgtccaggatgggaatttgcaaaggcagagatgttactgatcgtccatcattttgttagaaacttcagcagctttttcccagtcgacccaaatgaaaaaatttcaggagatccattccctcctctccctaccaatggattttctatgaaactttttcccagatcctag

SEQ ID NO: 18 - DNA, 1506 bp, unidentified
  source 1..1506: mol_type = other DNA; note = T9H4 reading frame nucleotide sequence
atggattccttaagttttctaaaaagcatggaagcgaaattcggccaagtcatacaccgggatcagtcttccagtactgctcttctgtccctcgcattcacagctgctcttgccatttttcttgtgttgctctttcgatttaaaagccggccctctactaatttccctccaggaaattttggcttccctttcattggagagacgatacagttcttgcgggcacttcgatcagaatcgcctcatatgttttttgatgagagattgaagaaatttgggcgtgtattcaagacgtcattaactgggcatcccacagctgtgttctgcgggcctgcgggaaaccggtttatttactcgaatgagcacaagctggtgcagtcgtctgggcccaactccttcgtcaaactggttgggcagcaatccatcgtgaccaaaacaggagaggagcaccgcatctttcgtggtgtcctgaacgagtttctggggcctcatgccttacagagttatacgcctaaaatgagttccaaaatccaggagaatatcaataagcattggaagggtaaagatgaagtgaacatgcttccttcgataagacagctcgtcttctccatttcaagcagcttgttttttgatattaatgatgaggatcaacaggaacaacttaaaactctgttagaaactattcttgttggaactttgtcggttcccctcgacattccaggatctaattttcgtaaagctcttcgggcgcgttccaagctggatgaaattctgtctcgtttaatcgaaagcagaagaaaagatatgcgttctgggatagcttctaccagtaaaaatctactgtcggtgctgctcgccttcaaagatgaaagagggaatccattgacggacacggagatcctcgacaacttttcttttatgcttcacgcctcatacgacaccaccgtttcgcccacggtttgtatatttaagctgctctccgccaatccagaatgctatgaaaaagtagttcaagaacaattgggaatacttggcaataaaaaggacggtgaagaaatctgttggaacgatctgaaagctatgaaatatacatggcaagcagctcaagaaacaatgaggcttttccctccagcgtttggatcatttcgcaaggtcatcgccgatattcttcatgatggctatataattcccaaaggatggaaagctatggtgacaaattacagtacaagtaggaaagaagagtacttcgatgaaccagacaaattcaagccttcaagatttggggaaggaaagtatgtggctccgtacacgttcttacctttcggggcaggaatacgcatatgcccaggatgggagttcgctaagttggagatgttactgttcatccatcattttgtcaaaaatttcagcggatacctcccacttgacaccaaggaaaagatttccggagatccattccctcctctccccaaaaatggatttcccattaaactatttcccagaacctaa

SEQ ID NO: 19 - DNA, 1500 bp, unidentified
  source 1..1500: mol_type = other DNA; note = T9H5 reading frame nucleotide sequence
atggatcgcttcaatttgctgagaggcatagtttcaaatttaggggaagtcattcaactggattcttcccctgcttttatttcccttaccctcgcagctatccttggcattattgtcctctttatcttccgttataatcaccgatcttctgttaaacttccccctggaaatttaggcttccccttcattggggagaccataccattcttgcgggcccttcgatcagaaacccctcaaacattttttgatgggagaatgaagaaattcggtcctgttttcctgacatcgctaattgggcatcccacagttgtattctgcgggcctgcgggaaatcgccttcttctctccaacgaggacaaactggtaaacatgacatcgcccaagtcttccagaaaagtgtttgggcagaattccattgtgaccaaaagaggcgaggagcatcgcatcttccgtgctgcacttacccgttttttgcgtccccaagccatacagagttatattggtagaatgaattccaaagtcgaacgtcatatcaacgaaaaatggaagggaaaagacgaagtgaaggcgcttcctttgataagagacctcatcttttccattgcaagcagtctgtttttcgatataaatgatgagcaccaacagaagcgacttcatcatctgttggaaaccgttcttatgggaagtatgtctgttccgctcgactttccaggaactccttttcgtaaagctgttcaggcgcgatcaaagctggatgaaattctttcttgtttaataaaaagcagaagaaacgatctccgttcgggcatagcttctgaagatcaagatcttctctctgtgttgctcaccttcaaagatgaaagaggaaatccactcgccgacaacgagatcctggacaacttttctgttatacttcatgcctcgtatgacaccactgtttcacccactgttttgctatttaagttcctcttctccaattctgaatgctatgaaaaagtagttcaagagcaattgggaatccatggcaataaaaaggagggggaagaaatcaattggaacgatctgaaagctatgaaatatacatggcaagtagttcaggaaacaatgaggattttccctccagcttttggagcttttcgccaagctatcaccgacattcactacgatggctatacagttccaaagggatacaatatattatggacaccttatgctacacatgtgaaagaagagtacttcaatgaagcggacaagttcatgccttcaagattcgaggaaggcaaatatgttaccccttacacatacttgccattcggagcaggcttgcgcgtatgtccaggatgggaatttgcaaaggcagagatgttactgatcgtccatcattttgttagaaacttcagcagctttttcccagtcgacccaaatgaaaaaatttcaggagatccattccctcctctccctaccaatggattttctatgaaactttttcccagatcctag

SEQ ID NO: 20 - DNA, 1506 bp, unidentified
  source 1..1506: mol_type = other DNA; note = T9H6 reading frame nucleotide sequence
atggattccttcagttttctaaaaagcatggaagcgaaattcggccaagtcatacaccgggatcagtcttccagtactgctcttctgtccctcgcattcacagctgctgttgccatttttcttgtgttgctctttcgatttaaaagccggccttctactaatttccctccaggaaattttggcttccctttcattggagagacgatacagttcttgcgggcacttcgatcagaatcgcctcatatgttttttgatgagagattgaagaagttcgggcgtgtattcaagacgtcattaactgggcaccccacagctgtgttctgcgggcctgcgggaaaccggtttatttactcgaatgagcacaagctggtgcagtcgtctgggcccaactcctttgtcaaactggttgggcagcaatccatcgtgaccaaaacaggagaggagcaccgcatctttcgtggtgtcctgaacgagtttctggggcctcatgccttacagagttatacgcctaaaatgagttccaaaatccaggagaatatcaataagcattggaagggtaaagatgaagtgaacatgcttccttcgataagacagctcgtcttctccatttcaagcagcttgttttttgatattaatgatgaggatcaacaggaacaacttaaaactcttttagaaactattcttgtgggaactttgtcggttcccctcgacattccaggatctaattttcgtaaagctcttcgggcgcgttccaagctggatgaaattctgtctcgtttaatcgaaagcagaagaaaagatatgcgttctgggatagcttctaccagtaaaaatctactgtcggtgctgctcgccttcaaagatgaaagagggaatccattgacggacacggagatcctcgacaacttttcttttatgcttcacgcctcatacgacaccaccgtttcgcccacagtttgtatatttaagctgctctccgccaatccagaatgctatgaaaaagtagttcaagaacaattgggaatacttggcaataaaaaggacggtgaagaaatctgttggaacgatctgaaagctatgaaatatacatggcaagcagctcaagaaacaatgaggcttttccctccagcgtttggatcatttcgcaaggtcatcgccgatattcatcatgatggctatataattcccaaaggatggaaagctatggtgacaaattacagtacaagtaggaaagaagagtacttcgatgaaccagacaaattcaagccttcaagatttggggatggaaagtatgtggctccgtacacgttcttacctttcggggcaggcatacgcatatgcccaggatgggagttcgctaagttggagatgttactgttcatccatcattttgtcaaaaatttcagcggatacctcccacttgacaccaaggaaaagatttccggagatccattccctcctctccccaaaaatggatttcccattaaactatttcccagaacctaa

SEQ ID NO: 21 - DNA, 1500 bp, unidentified
  source 1..1500: mol_type = other DNA; note = T9H7 reading frame nucleotide sequence
atggatcgcttcaattttgtgagagacatagttgcaaatttaggggaagtaattcaactggagtcttcccctgctattatttcccttaccctcgcagctatccttggcattattcttctttttatcttccgttataataaccgatcctctgttaaacttccccctggaaatttaggcttccccttcattggggagaccataccattcttgcgggcgcttcgatcagaaacccctcaaacattttttgatgggagaatgaagaaattcggccctgttttcctgacttcgctaattgggcatcccacagttgtattctgcgggcctgcgggaaatcgccttcttctctccaacgaggacaaactagtaaacatgacatcgcccaagtcttccagaaaagtgtttgggcagaattccattgtgaccaaaagaggcgaggagcatcgcatcttccgtgctgcacttgcccgttttttgcgtccccaagccatacagagttatattggtagaatgaattccaaagtcgaacgtcatatcaacgaaaaatggaagggaaaagacgaagtgaaggcgcttcctttgataagatacctcatcttttccattgcaagcagtctgtttttcgatataaatgatgagcaccaacagaagcgacttcatcatctgttggaaaccgttcttatgggaagtatgtctgttccgctcgactttccaggaactccttttcgtaaagctgttcaggcgcgatcaaagctggatgaaattctttcttgtttgataaaaagcagaagaaacgatctccgttcgggcatagcttctgaagatcaagatcttctctctgtgttgctcaccttcaaagatgaaagaggaaatccactcgccgacaacgagatcctggacaacttttctgttatacttcatgcctcgtatgacaccactgtttcacccagtgttttgctatttaagttcctcttctccaatcctgaatgctatgaaaaagtagttcaagagcaattgggaatccatggcaataaaaaggagggggaagaaatcaattggaacgatctgaaagctatgaaatatacatggcaagtagttcaggaaacaatgaggattttccctccagcttttggagcttttcgccaagctatcaccgacgttcactacgatggctatacagttccaaagggatacaatatattatggacaccttatgctacacatgtgaaagaagagtacttcaatgaagcggacaagttcatgccttcaagattcgaggaaggcaaatatgttgccccttacacatacttgccattcggagcaggcttgcgcgtatgtccaggatgggaatttgcaaaggcagagatgttactgatcgtccatcattttgttagaaacttcagcagctttttcccagtcgacccaaatgaaaaaatttcaggagatccattccctcctctccctaccaatggattttctatgaaactttttcccagatcctag

SEQ ID NO: 22 - DNA, 1506 bp, unidentified
  source 1..1506: mol_type = other DNA; note = T9H8 reading frame nucleotide sequence
atggattccttcagttttctaaaaagcatggaagcgaaatttggccaagtcatccaccgggatcagtcttccagtactgttcttctgtccctcgcattcacagctgctgttgccatttttcttgtgttgctctttcgatttaaaagccggccctctactaatttccctccaggaaattttggcttccctttcattggagagacgatacagttcttgcgggcacttcgatcagaatcgcctcataggttttttgatgagagattgaagaaatttgggaatgtattcaagacgtcattaactgggcatcccacagctgtgttctgcgggcctgcgggaaaccggtttatttactcgaatgagcacaagctggtgcagtcgtctgggcccaactccttcgtcaaactggttgggcagcaatccatcgtgaccaaaacaggagaggagcatcgcatctttcgtggtgtcctgaacgagtttctggggcctcatgccttacagagttatacgcctaaaatgagttccaaaatccaggagaatatcaataagcattggaagggtaaagatgaagtgaacatgcttccttcgataagacagctcgtcttctccatttcaagcagcttgttttttgatattaatgatgaggatcaacaggaacaacttaaaactcttttagaaactattcttgttggaactttgtcggttcccctcgacattccaggatctaattttcgtaaagctcttcgggcgcgttccaagctggatgaaattctgtctcgtttaatcgaaagcagaagaaaagatatgcgttctgggatagcttctaccagtaaaaatctactgtcggtgctgctcgccttcaaagatgaaagagggaatccattgacggacacggagatcctcgacaacttttcttttatgcttcacgcctcatacgacaccaccgtttcgcccacggtttgtatatttaagctgctctccgccaatccagaatgctatgaaaaagtagttcaagaacaattgggaatacttggcaataaaaaggacggtgaagaaatctgttggaacgatctgaaagctatgaaatatacatggcaagcagctcaagaaacaatgaggcttttccctccagcgtttggatcatttcgcaaggtcatcgccgatattcatcatgatggctatataattcccaaaggatggaaagctatggtgacaaattacagtacaagtaggaaagaagagtacttcgatgaaccagacaaattcaagccttcaagatttggggatggaaagtatgtggctccgtacacgttcttacctttcggggcaggcatacgcatatgcccaggatgggagttcgctaagttggagatgttactgttcatccatcattttgtcaaaaatttcagcggatacctcccacttgacaccaaggaaaagatttccggagatccattccctcctctccccaaaaatggatttcccattaaactatttcccagaacctaa

SEQ ID NO: 23 - DNA, 1500 bp, unidentified
  source 1..1500: mol_type = other DNA; note = T9H9 reading frame nucleotide sequence
atggatcgcttcaatttgctgagaggcatagtttcaaatttaggggaagtcattcaactggactcttcccctgctattatttcccttaccctcgcagctatccttggcattattgtcctctttatcttccgttataatcaccgatcttctgttaaacttccccctggaaatttaggcttccccttcattggggagaccataccattcttgcaggcgcttcgatcagaaacccctcaaacattttttgatgggagaatgaagaaattcggtcctgttttcctgacatcgctaattgggcatcccacagttgtattctgcgggcctgcgggaaatcgccttcttctctccaacgaggacaaactggtaaacatgacatcgcccaagtcttccagaaaagtgtttgggcagaattccattgtgaccaaaagaggcgaggagcatcgcatcttccgtgctgcacttacccgttttttgcgtccccaagccatacagagttatattggtagaatgaattccaaagtcgaacgtcatatcaacgaaaaatggaagggaaaagacgaagtgaaggcgcttcctttgataagagacctcatcttttccattgcaagcagtctgtttttcgatataaatgatgagcaccaacagaagcgacttcatcatctgttggaaaccgttcttatgggaagtatgtctgttccgctcgactttccaggaactccttttcgtaaagctgttcaggcgcgatcaaagctggatgaagttctttcttgtttgataaaaagcagaagaaacgatctccgttcgggcatagcttctgaagatcaagatcttctctctgtgttgctcaccttcaaagatgaaagaggaaatccactcgccgacaacgagatcctggacaacttttctgttatacttcatgcctcgtatgacaccactgtttcacccactgttttgctatttaagttcctcttctccaatcctgaatgctatgaaaaagtagttcaagagcaattgggaatccatggcaataaaaaggagggggaagaaatcaattggaacgatctgaaagctatgaaatatacatggcaagtagttcaggaaacaatgaggattttccctccagcttttggagcttttcgccaagctatcaccgatattcactacgatggctatacagttccaaagggatacaatatattatggacaccttatgctacacatgtgaaagaagagtacttcaatgaagcggacaagttcatgccttcaagattcgaggaaggcaaatatgttaccccttacacatacttgccattcggagcaggcttgcgcgtatgtccaggatgggaatttgcaaaggcagagatgttactgatcgtccatcattttgttagaaacttcagcagctttttcccagtcgacccaactgaaaaaatttcaggagatccattccctcctctccctaccaatggattttctatgaaactttttcccagatcctag

SEQ ID NO: 24 - DNA, 1479 bp, unidentified
  source 1..1479: mol_type = other DNA; note = T9H10 reading frame nucleotide sequence
atggatagcttcaatttcccgagagggggagtcattcagctgggttattcccctgctattctttcccttaccctcgcacctattcttgccattctcctcctcttcttcttccgttacactcaccgatcctctgataaacttcccccgggaaatttagggtttcctttcattggggagactatacagttaatgcgggcacttcgaacagaaacacctcagacgtttttcgatgagagagtgaagaagttcggtcatgttttcaagacttcgctcattgggtatcccacagttgtactgagtggacctgcgggaaacaggttacttctgtcgaacgaggagaagctggtgcattcgtcatcgcccaagtctaccctgaaattgttcgggcaggattctgttctgaccaaaagaggcgaggagcatcgtatcttccgtgccgcacttgcccgcttcttgcgaccccaagctttacagggttatgttgccaaaatgaattcagaaattcaacatcatatgaatcaaaaatggaagggaaaacatcaagtgaaggtgcttcctttggtaagagcgcttatcttcaacattgcaagcagcttttttttcggtataactgacgaacacctacaggaacgacttcataaccttttggaagctattcttctgggaagtatgtctgttccgctcgactttccaggcactcgttttcgtaaagctcttgaggcgcggtcgaagctggacgaaattctttcttctttgataaaaaagagaagaagcgatcttctgcgttcaacttctgacaatcaagatcttctttctgtgttgctcaccttcaaagatgaaagagggaatccactgacggacaaggagatccttgacaatttttctgtcatgcttcatggctcgtatgagaccagtgtttcacccacggttttggtgtttaagcttctcttctcaaatcctgattgctatgagaaagtagttcaagagcaattgggaatcctgtgcaataaaaaggagggagaagaaatcagctggaacgatctgaaaactatgaaatatacatggcaagttgtgcaggaaactatgaggatgttccctccagtttttggatcgtatcgcaaggctatcaccgatatccattatgatgggtatacaattccaaaaggatggaaaatattctggtcaccttatactacacacgggaaagaagagtacttcaatgaagcggacaagttcatgccttcaagattcgaggaaggcaaatatgttgctccttacacattcttgccattcggagcaggtgtccgcgtatgtccagggtgggaatttgcaaagaccgagatattactgttcgtccatcattttgttagaactttcagcagctacatcccaattgaccccaaagagaaaatttcaggggatccatttcctcctctgcctaccaatggattttccatgaaacttttttccagatcttaa

SEQ ID NO: 25 - DNA, 1479 bp, unidentified
  source 1..1479: mol_type = other DNA; note = T9H11 reading frame nucleotide sequence
atggatagcttcaatttcccgagagggggagtcattcagctgggttattcccctgctattctttcccttaccctcgcacctattcttgccattctcctcctcttcttcttccgttacactcaccgatcctctgataaacttcccccgggaaatttagggtttcctttcattggggagactatacagttaatgcgggcacttcgaacagaaacacctcagacgtttttcgatgagagagtgaagaagttcggtcatgttttcaagacttcgctcattgggtatcccacagttgtactgagtggacctgcgggaaacaggttacttctgtcgaacgaggagaagctggtgcattcgtcatcgcccaagtctaccctgaaattgttcgggcaggattctgttctgaccaaaagaggcgaggagcatcgtatcttccgtgccgcacttgcccgcttcttgcgaccccaagctttacagggttatgttgccaaaatgaattcagaaattcaacatcatatgaatcaaaaatggaagggaaaacatcaagtgaaggtgcttcctttggtaagagcgcttatcttcaacattgcaagcagcttttttttcggtataactgacgaacacctacaggaacgacttcataaccttttggaagctattcttctgggaagtatgtctgttccgctcgactttccaggcactcgttttcgtaaagctcttgaggcgcggtcgaagctggacgaaattctttcttctttgataaaaaagagaagaagcgatcttctgcgttcaacttctgacaatcaagatcttctttctgtgttgctcaccttcaaagatgaaagagggaatccactgacggacaaggagatccttgacaatttttctgtcatgcttcatggctcgtatgagaccagtgtttcacccacggttttggtgtttaagcttctcttctcaaatcctgattgctatgagaaagtagttcaagagcaattgggaatcctgtgcaataaaaaggagggagaagaaatcagctggaacgatctgaaaactatgaaatatacatggcaagttgtgcaggaaactatgaggatgttccctccagtttttggatcgtatcgcaaggctatcaccgatatccattatgatgggtatacaattccaaaaggatggaatatattctggtcaccttatactacacacgggaaagaagaatacttcaatgaagcggacaagttcatgccttcgagattcgaggaaggcaaatatgttgctccttacacattcttgccattcggagcaggtctgcgcgtatgtccaggatgggaatttgcaaagaccgagatattactgttcgtccatcattttgttacaactttcagcagctacatcccaattgaccccatagagaaaatttcaggggatccattccctcctctgcccaccgatggattttccatgaaactttttaccagatcttaa

SEQ ID NO: 26 - DNA, 1506 bp, unidentified
  source 1..1506: mol_type = other DNA; note = T9H12 reading frame nucleotide sequence
atggattccttcagttttctaaaaagcatggaagcgaaattcggccaagtcatacaccgggatcagtcttccagtactgctcttctgtccctcgcattcacagctgctgttgccatttttcttgtgttgctctttcgatttaaaagccggccttctactaatttccctccaggaaattttggcttccctttcattggagagacgatacagttcttgcgggcacttcgatcagaatcgcctcatatgttttttgatgagagattgaagaaatttgggcgtgtattcaagacgtcattaactgggcatcccacagctgtgttctgcgggcctgcgggaaaccggtttatttactcgaatgagcacaagctggtgcagtcgtctgggcccaactcctttgtcaaactggttgggcagcaatccatcgtgaccaaaacaggagaggagcaccgcatctttcgtggtgtcctgaacgagtttctggggcctcatgccttacagagttatacgcctaaaatgagttccaaaatccaggagaatatcaataagcattggaagggtaaagatgaagtgaacatgcttccttcgataagacagctcgtcttctccatttcaagcagcttgttttttgatattaatgatgaggatcaacaggaacaacttaaaactcttttagaaactattcttgtgggaactttgtcggttcccctcgacattccaggatctaattttcgtaaagctcttcgggcgcgttccaagctggatgaaattctgtctcgtttaatcgaaagcagaagaaaagatatgcgttctgggatagcttctaccagtaaaaatctactgtcggtgctgctcgccttcaaagatgaaagagggaatccattgacggacacggagatcctcgacaacttttcttttatgcttcacgcctcatacgacaccaccgtttcgcccacagtttgtatatttaagctgctctccgccaatccagaatgctatgaaaaagtagttcaagagcaattgggaatacatggcaataaaaaggagggggaagaaatcaattggaacgatctgaaagctatgaaatatacatggcaagcagctcaagaaacaatgaggcttttccctccagcgtttggatcatttcgcaaggtcatcgccgatattcatcatgatggctatataattcccaaaggatggaaagctatggtgacaaattacagtacaagtaggaaagaagagtacttcgatgaaccagacaaattcaagccttcaagatttggggatggaaagtatgtggctccgtacacgttcttacctttcggggcaggcatacgcatatgcccaggatgggagttcgctaagttggagatgttactgttcatccatcattttgtcaaaaatttcagcggatacctcccacttgacaccaaggaaaagatttccggagatccattccctcctctccccaaaaatggatttcccattaaactatttcccagaacctaa

SEQ ID NO: 27 - DNA, 1476 bp, unidentified
  source 1..1476: mol_type = other DNA; note = T9H13 reading frame nucleotide sequence
atgaataccttcagtttcctgcctccaaatttcctcgggttcattcaactccagtctattctattccttacccttcttgcccttcttcttctctgcctcttccgatataaaaccccgtcctctgctgttaaacttccccctggaaacttagggttccctttcattggggagaccataccattcttgagggcacttcactcagaaacaccgcaaacctttttcgatgagagaatgaagagattcggtaatgttttcgtgacttcgctaattggacagccaatagttgtactctgcgggcctgccggaaaccgcttactactctccaacgaagacaagctggtggaaatgtcaccacccaagttttcgctgaagctgatcggccaggattcccttctgtccaaaagagaagacgagcatcgcaccctacgcgctgcactcgctcgctttctgcgaccccaagcccttcagagttatatgggtataatgagttcagaaatcgaacagcatatcaatgaaaaatggaaggtaaaagatgaagtgaagatgcttcctttgataagaggacttatcttctccattgcaaccaccttgtttttcgatatcaatgatgagcacctcaaggatcgccttcatcaccttttggaaactattcttgtgggaactgtgtctcttccgctcgacttcccaggaacttcttttcgtaaagctgttgaggcgcggtcgaagctcgatgaaattctttcttctttaataaaaagcagaagaagcgatctgcattcaggcatagtttctgatggtcaagatctgctcacagtcttgctcaccttcaaagacgaaagagggaattcactcgccgataacgagatcctcgacaacttttctcttatgcttcacgcctcctatgagaccagtgtttcaccaacggttttgatgtttaagctgctgtcctccaatcctgaatgttatgacaaactagttcaagagcaattgggaatacttgccaataaaaaggagggagaagacatcagctggaaggatgtgaaagctatgaaatatacatggcaagtagttcaggaaacaatgaggattttccctccagcttttggagcttttcgccaagctatcaccgacattcactacgatggctatacagttccaaagggatacaatatattatggacaccttatgctacacatgtgaaagaagagtacttcaatgaagcggacaagttcatgccttcaagattcgaggaaggcaaatatgttgccccttacacatacttgccattcggagccggcttgcgcgtatgtccaggatgggaatttgcaaaggcagagatgttactgatcgtccatcattttgttagaaacttcagcagctttttcccagtcgacccaaatgaaaaaatttcaggagatccattccctcctctccctaccaatggattttccatgaaactttttcccagatcttaa

SEQ ID NO: 28 - DNA, 1476 bp, unidentified
  source 1..1476: mol_type = other DNA; note = T9H14 reading frame nucleotide sequence
atgaataccttcagtttcctgcctccaaatttcctcgggttcattcaactccagtctattctattccttacccttcttgcccttcttcttctctgcctcttccgatataaaaccccgtcctctgctgttaaacttccccctggaaacttagggttccctttcattggggagaccataccattcttgagggcacttcactcagaaacaccgcaaacctttttcgatgagagaatgaagagattcggtaatgttttcgtgacttcgctaattggacagccaatagttgtactctgcgggcctgccggaaaccgcttactactctccaacgaagacaagctggtggaaatgtcaccacccaagttttcgctgaagctgatcggccaggattcccttctgtccaaaagagaagacgagcatcgcaccctacgcgctgcactcgctcgctttctgcgaccccaagcccttcagagttatatgggtataatgagttcagaaatcgaacagcatatcaatgaaaaatggaaggtaaaagatgaagtgaagatgcttcctttgataagaggacttatcttctccattgcaaccaccttgtttttcgatatcaatgatgagcacctcaaggatcgccttcatcaccttttggaaactattcttgtgggaactgtgtctcttccgctcgacttcccaggaacttcttttcgtaaagctgttgaggcgcggtcgaagctcgatgaaattctttcttctttaataaaaagcagaagaagcgatctgcattcaggcatagtttctgatggtcaagatctgctcacagtcttgctcaccttcaaagacgaaagagggaattcactcgccgataacgagatcctcgacaacttttctcttatgcttcacgcctcctatgagaccagtgtttcaccaacggttttgatgtttaagctgctgtcctccaatcctgaatgttatgacaaactagttcaagagcaattgggaatacttgccaataaaaaggagggagaagacatcagctggaaggatgtgaaagctatgaaatatacatggcaagtagttcaggaaacaatgaggatattccctccaggttttggatcatatcgtaaggcgatcaccgatattgattatgatggttatacaattccaaaaggatggacaactttatggactccttatactacacatgggaaagaacagtacttccatgatcccgaacaattcaggccttcaagatttgaagaaggagaacgtgtagctccttacacattcttaccattcggagcaggcgcgcgcatatgtccaggatgggaattcgcaaagacagagatattactgttcgtccatcattttgttaaaaatttcagtagctaccacttagttgaccccaaggaaaaagtatcagggaatccattccctcctctccctaacaatggattttctctgaaagtatttcccagatcgtaa

SEQ ID NO: 29 - DNA, 1524 bp, unidentified
  source 1..1524: mol_type = other DNA; note = TOT reading frame nucleotide sequence
atggttcatgtgttgcacgtagtgaaaatggatagagttagagaaatatttaatggaagttcaggttctccagctggtattccccacagtgtgatcacagccggtgtgggtgccataataataattcttctgtcactactgctcctccgccgttctagtaaacggggcgactcctctcatcctcctgggaattcaggccttccattcattggggagacattatcattcaccaaggcttttaaatcgaacacgctggccgaattttttgaggagagggtgaagaaattcgggaatgtatttaagatttcaataatcgggcctcccacagtggtaatgtgcggcaatgagggaaaccggtttattttcgccaacgaggagaagctgatgcacctgtcgtggtccggtcgatatgcgaaaatccttggtggggaatccgtttccatgaagaggggagatgatcatcgcagtgtacgtgccgcattcgcagggtttttgagctctgcatcgctgcctgtttacataagtaaaatgagtgcacagatccaagatcatatcaacgaaaaatggaaaggaaaagatgtaattgctgtagttcctctggtaaaggagctcgtcttcaacgtttcctacaacttgtttttcagcataaatgatagcgaggaactgcatcgattgcataagattttcgaaactattgtggagggacatctttccatgccgatagaccttcccggattcacctttcatagagcacttcagggaagggcgaagctcaagaaagttttctcttctttaatagaaaggagaagaagcgatctgagctccggattggcatctgctaatcaggatctcatttctgttttactcacctacaaagatgatagggggtatacaatgacccacgacgagctcctcgacaactttctttcccttcttgaaggctcctatgattccatcaattcaccaatggcctgcatttttaagcttttgtatgacaatccagaatgctatgaaaaagtagttcaagagcaattggggatactttctggtaagaaggaaggacaagaaatctcgtggaaggatctgagatccatgaaatacacatggcaagtacttcaggaaacgctacgactgtatactcaagttgctggaatatttcgcaaagccatgactgacattcattatgatggtcacaccattcccaaagggtggcaacttctttgggcaaaccaaactacacatctgaacgacaaatatttcagtgagcctgaaaaattcatgccttccagattcgatgaagaaggaaacaatatgattccttactcattcgtaccatttggaggagggcggcggatgtgtccaggttgggaattcggaaagatggagatcttactctttgtccatcactttgttaaaacgttcagtggctttaccccaattgatccgaacgaaaaaattactgggaatccttttcctcatctccctgccaatggatttctaataaaacctattctcagatcctaa

SEQ ID NO: 30 - DNA, 53 bp, synthetic construct
  source 1..53: mol_type = other DNA; note = P1 primer sequence
gtatattctgcccaaattcgcgaatggattccttaagttttctaaaaagcatg

SEQ ID NO: 31 - DNA, 57 bp, synthetic construct
  source 1..57: mol_type = other DNA; note = P2 primer sequence
tgaaaccagagttaaaggcctcgagttaggttctgggaaatagtttaatgggaaatc

SEQ ID NO: 32 - DNA, 50 bp, synthetic construct
  source 1..50: mol_type = other DNA; note = P3 primer sequence
gtatattctgcccaaattcgcgaatggattgcttcaattttctaacaagc

SEQ ID NO: 33 - DNA, 51 bp, synthetic construct
  source 1..51: mol_type = other DNA; note = P4 primer sequence
tgaaaccagagttaaaggcctcgagttaggttctgggaaggagttttatgg

SEQ ID NO: 34 - DNA, 44 bp, synthetic construct
  source 1..44: mol_type = other DNA; note = P5 primer sequence
gtatattctgcccaaattcgcgaatggatcgcttcaatttgctg

SEQ ID NO: 35 - DNA, 56 bp, synthetic construct
  source 1..56: mol_type = other DNA; note = P6 primer sequence
tgaaaccagagttaaaggcctcgagctaggatctgggaaaaagtttcatagaaaat